European Patent Application EP 4 245 322 A1, published September 20, 2023. Title: TREATMENT OF MESOTHELIOMA BY ADMINISTRATION OF ANTI-B7-H3 ANTIBODY-DRUG CONJUGATE. Applicant: DAIICHI SANKYO COMPANY, LIMITED. Application 21891940.5. The sequence listing filed with the application follows.

SEQUENCE LISTING (13 sequences)

SEQ ID NO: 1 - protein, 534 aa, Homo sapiens
MLRRRGSPGMGVHVGAALGALWFCLTGALEVQVPEDPVVALVGTDATLCCSFSPEPGFSLAQLNLIWQLTDTKQLVHSFAEGQDQGSAYANRTALFPDLLAQGNASLRLQRVRVADEGSFTCFVSIRDFGSAAVSLQVAAPYSKPSMTLEPNKDLRPGDTVTITCSSYQGYPEAEVFWQDGQGVPLTGNVTTSQMANEQGLFDVHSILRVVLGANGTYSCLVRNPVLQQDAHSSVTITPQRSPTGAVEVQVPEDPVVALVGTDATLRCSFSPEPGFSLAQLNLIWQLTDTKQLVHSFTEGRDQGSAYANRTALFPDLLAQGNASLRLQRVRVADEGSFTCFVSIRDFGSAAVSLQVAAPYSKPSMTLEPNKDLRPGDTVTITCSSYRGYPEAEVFWQDGQGVPLTGNVTTSQMANEQGLFDVHSVLRVVLGANGTYSCLVRNPVLQQDAHGSVTITGQPMTFPPEALWVTVGLSVCLIALLVALAFVCWRKIKQSCEEENAGAEDQDGEGEGSKTALQPLKHSDSKEDDGQEIA

SEQ ID NO: 2 - protein, 316 aa, Homo sapiens
MLRRRGSPGMGVHVGAALGALWFCLTGALEVQVPEDPVVALVGTDATLCCSFSPEPGFSLAQLNLIWQLTDTKQLVHSFAEGQDQGSAYANRTALFPDLLAQGNASLRLQRVRVADEGSFTCFVSIRDFGSAAVSLQVAAPYSKPSMTLEPNKDLRPGDTVTITCSSYRGYPEAEVFWQDGQGVPLTGNVTTSQMANEQGLFDVHSVLRVVLGANGTYSCLVRNPVLQQDAHGSVTITGQPMTFPPEALWVTVGLSVCLIALLVALAFVCWRKIKQSCEEENAGAEDQDGEGEGSKTALQPLKHSDSKEDDGQEIA

SEQ ID NO: 3 - protein, 471 aa, Artificial Sequence
  Heavy chain of anti-B7-H3 antibody
MKHLWFFLLLVAAPRWVLSQVQLVQSGAEVKKPGSSVKVSCKASGYTFTNYVMHWVRQAPGQGLEWMGYINPYNDDVKYNEKFKGRVTITADESTSTAYMELSSLRSEDTAVYYCARWGYYGSPLYYFDYWGQGTLVTVSSASTKGPSVFPLAPSSKSTSGGTAALGCLVKDYFPEPVTVSWNSGALTSGVHTFPAVLQSSGLYSLSSVVTVPSSSLGTQTYICNVNHKPSNTKVDKRVEPKSCDKTHTCPPCPAPELLGGPSVFLFPPKPKDTLMISRTPEVTCVVVDVSHEDPEVKFNWYVDGVEVHNAKTKPREEQYNSTYRVVSVLTVLHQDWLNGKEYKCKVSNKALPAPIEKTISKAKGQPREPQVYTLPPSREEMTKNQVSLTCLVKGFYPSDIAVEWESNGQPENNYKTTPPVLDSDGSFFLYSKLTVDKSRWQQGNVFSCSVMHEALHNHYTQKSLSLSPGK

SEQ ID NO: 4 - protein, 233 aa, Artificial Sequence
  Light chain of anti-B7-H3 antibody
MVLQTQVFISLLLWISGAYGEIVLTQSPATLSLSPGERATLSCRASSRLIYMHWYQQKPGQAPRPLIYATSNLASGIPARFSGSGSGTDFTLTISSLEPEDFAVYYCQQWNSNPPTFGQGTKVEIKRTVAAPSVFIFPPSDEQLKSGTASVVCLLNNFYPREAKVQWKVDNALQSGNSQESVTEQDSKDSTYSLSSTLTLSKADYEKHKVYACEVTHQGLSSPVTKSFNRGEC

SEQ ID NO: 5 - protein, 471 aa, Artificial Sequence
  Heavy chain of anti-B7-H3 antibody
MKHLWFFLLLVAAPRWVLSQVQLVQSGAEVKKPGSSVKVSCKASGYTFTNYVMHWVRQAPGQGLEWIGYINPYNDDVKYNEKFKGRVTITADESTSTAYMELSSLRSEDTAVYYCARWGYYGSPLYYFDYWGQGTLVTVSSASTKGPSVFPLAPSSKSTSGGTAALGCLVKDYFPEPVTVSWNSGALTSGVHTFPAVLQSSGLYSLSSVVTVPSSSLGTQTYICNVNHKPSNTKVDKRVEPKSCDKTHTCPPCPAPELLGGPSVFLFPPKPKDTLMISRTPEVTCVVVDVSHEDPEVKFNWYVDGVEVHNAKTKPREEQYNSTYRVVSVLTVLHQDWLNGKEYKCKVSNKALPAPIEKTISKAKGQPREPQVYTLPPSREEMTKNQVSLTCLVKGFYPSDIAVEWESNGQPENNYKTTPPVLDSDGSFFLYSKLTVDKSRWQQGNVFSCSVMHEALHNHYTQKSLSLSPGK

SEQ ID NO: 6 - protein, 471 aa, Artificial Sequence
  Heavy chain of anti-B7-H3 antibody
MKHLWFFLLLVAAPRWVLSEVQLVQSGAEVKKPGSSVKVSCKASGYTFTNYVMHWVKQAPGQGLEWIGYINPYNDDVKYNEKFKGKATITADESTSTAYMELSSLRSEDTAVYYCARWGYYGSPLYYFDYWGQGTLVTVSSASTKGPSVFPLAPSSKSTSGGTAALGCLVKDYFPEPVTVSWNSGALTSGVHTFPAVLQSSGLYSLSSVVTVPSSSLGTQTYICNVNHKPSNTKVDKRVEPKSCDKTHTCPPCPAPELLGGPSVFLFPPKPKDTLMISRTPEVTCVVVDVSHEDPEVKFNWYVDGVEVHNAKTKPREEQYNSTYRVVSVLTVLHQDWLNGKEYKCKVSNKALPAPIEKTISKAKGQPREPQVYTLPPSREEMTKNQVSLTCLVKGFYPSDIAVEWESNGQPENNYKTTPPVLDSDGSFFLYSKLTVDKSRWQQGNVFSCSVMHEALHNHYTQKSLSLSPGK

SEQ ID NO: 7 - protein, 471 aa, Artificial Sequence
  Heavy chain of anti-B7-H3 antibody
MKHLWFFLLLVAAPRWVLSEVQLVQSGAEVKKPGSSVKVSCKASGYTFTNYVMHWVKQAPGQGLEWIGYINPYNDDVKYNEKFKGKATQTSDKSTSTAYMELSSLRSEDTAVYYCARWGYYGSPLYYFDYWGQGTLVTVSSASTKGPSVFPLAPSSKSTSGGTAALGCLVKDYFPEPVTVSWNSGALTSGVHTFPAVLQSSGLYSLSSVVTVPSSSLGTQTYICNVNHKPSNTKVDKRVEPKSCDKTHTCPPCPAPELLGGPSVFLFPPKPKDTLMISRTPEVTCVVVDVSHEDPEVKFNWYVDGVEVHNAKTKPREEQYNSTYRVVSVLTVLHQDWLNGKEYKCKVSNKALPAPIEKTISKAKGQPREPQVYTLPPSREEMTKNQVSLTCLVKGFYPSDIAVEWESNGQPENNYKTTPPVLDSDGSFFLYSKLTVDKSRWQQGNVFSCSVMHEALHNHYTQKSLSLSPGK

SEQ ID NO: 8 - protein, 233 aa, Artificial Sequence
  Light chain of anti-B7-H3 antibody
MVLQTQVFISLLLWISGAYGEIVLTQSPATLSLSPGERATLSCRASSRLIYMHWYQQKPGQAPRLLIYATSNLASGIPARFSGSGSGTDFTLTISRLEPEDFAVYYCQQWNSNPPTFGQGTKVEIKRTVAAPSVFIFPPSDEQLKSGTASVVCLLNNFYPREAKVQWKVDNALQSGNSQESVTEQDSKDSTYSLSSTLTLSKADYEKHKVYACEVTHQGLSSPVTKSFNRGEC

SEQ ID NO: 9 - protein, 233 aa, Artificial Sequence
  Light chain of anti-B7-H3 antibody
MVLQTQVFISLLLWISGAYGEIVLTQSPATLSLSPGERATLSCRASSRLIYMHWYQQKPGQAPRLWIYATSNLASGIPARFSGSGSGTDYTLTISRLEPEDFAVYYCQQWNSNPPTFGQGTKVEIKRTVAAPSVFIFPPSDEQLKSGTASVVCLLNNFYPREAKVQWKVDNALQSGNSQESVTEQDSKDSTYSLSSTLTLSKADYEKHKVYACEVTHQGLSSPVTKSFNRGEC

SEQ ID NO: 10 - protein, 233 aa, Artificial Sequence
  Light chain of anti-B7-H3 antibody
MVLQTQVFISLLLWISGAYGQIVLSQSPATLSLSPGERATLTCRASSRLIYMHWYQQKPGSAPKLWIYATSNLASGIPARFSGSGSGTSYTLTISRLEPEDFAVYYCQQWNSNPPTFGQGTKVEIKRTVAAPSVFIFPPSDEQLKSGTASVVCLLNNFYPREAKVQWKVDNALQSGNSQESVTEQDSKDSTYSLSSTLTLSKADYEKHKVYACEVTHQGLSSPVTKSFNRGEC

SEQ ID NO: 11 - protein, 233 aa, Artificial Sequence
  Humanized light chain of M30
MVLQTQVFISLLLWISGAYGQIVLSQSPATLSLSPGERATLTCRASSRLIYMHWYQQKPGSAPKPWIYATSNLASGIPARFSGSGSGTSYTLTISRLEPEDFAVYYCQQWNSNPPTFGQGTKVEIKRTVAAPSVFIFPPSDEQLKSGTASVVCLLNNFYPREAKVQWKVDNALQSGNSQESVTEQDSKDSTYSLSSTLTLSKADYEKHKVYACEVTHQGLSSPVTKSFNRGEC

SEQ ID NO: 12 - protein, 233 aa, Artificial Sequence
  Light chain of anti-B7-H3 antibody
MVLQTQVFISLLLWISGAYGEIVLTQSPATLSLSPGERATLSCRASSRLIYMHWYQQKPGQAPRPLIYATSNLASGIPARFSGSGSGTDFTLTISRLEPEDFAVYYCQQWNSNPPTFGQGTKVEIKRTVAAPSVFIFPPSDEQLKSGTASVVCLLNNFYPREAKVQWKVDNALQSGNSQESVTEQDSKDSTYSLSSTLTLSKADYEKHKVYACEVTHQGLSSPVTKSFNRGEC

SEQ ID NO: 13 - protein, 233 aa, Artificial Sequence
  Light chain of anti-B7-H3 antibody
MVLQTQVFISLLLWISGAYGEIVLTQSPATLSLSPGERATLSCRASSRLIYMHWYQQKPGQAPRPLIYATSNLASGIPARFSGSGSGTDYTLTISRLEPEDFAVYYCQQWNSNPPTFGQGTKVEIKRTVAAPSVFIFPPSDEQLKSGTASVVCLLNNFYPREAKVQWKVDNALQSGNSQESVTEQDSKDSTYSLSSTLTLSKADYEKHKVYACEVTHQGLSSPVTKSFNRGEC